European Patent Application EP 4 545 092 A1, published April 30, 2025. Title: COMPUTATIONALLY DESIGNED BINDERS FOR IMMUNE CELL THERAPIES. Applicant: Technische Universität München. The sequence listing filed with the application follows.

SEQUENCE LISTING (92 sequences)

SEQ ID NO: 1 - protein, 63 aa, synthetic construct
SLDEAKKLLQEAEKLARKLNDRMELAYVEFLKHILETAKKQNDKRTIESVRDMARDALEELQS

SEQ ID NO: 2 - protein, 62 aa, synthetic construct
DHWEEVFRWALEHLQEATQQNDPQKAKKILEEAHKWLRRELSEEEARAVVRWLKQLVDRELS

SEQ ID NO: 3 - protein, 63 aa, synthetic construct
SEKMKNIQELLAEADKYLEKAKAAKTKEEAKAYLRKAAEKLLQSPLSGLQEVASRILEKLEKE

SEQ ID NO: 4 - protein, 63 aa, synthetic construct
MKSKLKSYSEAALLYLTGGKEKLELAEKLLSEMYDLLGDEAAKERAKKNIEELRKEEEEKLKK

SEQ ID NO: 5 - protein, 63 aa, synthetic construct
MEEEKETSEYMRQTLHETLVAMGLDELALELYSEAKEKGWNLQEIVDMNDKRLAAIAAEEAAA

SEQ ID NO: 6 - protein, 63 aa, synthetic construct
GDRNIARMMNFIKEKLAELRADPAGAPKAEAIEKRMEEISKALKEDFSTGLVLLNELYKELLD

SEQ ID NO: 7 - protein, 63 aa, synthetic construct
MENLINEYKNAADELYKKALEKNPDLAFEIIMEVIDLEEKKETVTEEDIKEKIKKLKERLALL

SEQ ID NO: 8 - protein, 63 aa, synthetic construct
LEEKLKEAEKKLKETIKSVGVSQETLDEINNIIKSQHAKLALNGVGEGEYVKVLNELIEKIKK

SEQ ID NO: 9 - protein, 63 aa, synthetic construct
DLMEQIARSLRDEFVARLEAEGLGPELIAEARERLEKLLSVLEASTLKLLLAEVEEWVARKLA

SEQ ID NO: 10 - protein, 63 aa, synthetic construct
MREEELKKRREEVLKKVEELTKLGGKDLEFKAELAELLEKVEEGDEEALKELDRLLDEAFKKL

SEQ ID NO: 11 - protein, 63 aa, synthetic construct
SIPSELQLLALKLLDLTDKLAKDPSVAKEAKELRDKIIEAIRSGDEKELLEIKKELDAFLASK

SEQ ID NO: 12 - protein, 63 aa, synthetic construct
SDATRQLESLLDQIEALLAAGDLEAATQQWQQLVALLGDLSAEDLEKLLPRIQAAQQAFMALP

SEQ ID NO: 13 - protein, 62 aa, synthetic construct
MDKEKEIEEQAKKLKEIAEKLKKELGADESEVNLIVELAVKRIELGMSFEDALKEAIEQLKK

SEQ ID NO: 14 - protein, 62 aa, synthetic construct
NKAEEEREKLKEEIKEIIEELIKKNPSLTQETIEKINSTLENLILAGASKEDIIKALKKEIE

SEQ ID NO: 15 - protein, 62 aa, synthetic construct
ADELQEKLNKLNALMLKYRNSRATEIYYNLALKLEELAKTGTEETKEKVKKAEEKLKEYEAK

SEQ ID NO: 16 - protein, 62 aa, synthetic construct
SSAEYQALLEQKRLEARRLLAEALLKGSEELKEKLKEKLKEWREEGFPEELIKELEEELEKA

SEQ ID NO: 17 - protein, 62 aa, synthetic construct
LLEEFKKELDELLEKIKSGEVTEEDLLKKTEEAIEEVKKLPNAEKYQTELKRLVAEALLKLS

SEQ ID NO: 18 - protein, 62 aa, synthetic construct
EEEEQKKNLLKQKLKIKAEFLIEKTGDKEKVLELEKKYIEALDSGKNKEEAEKLLKEMESLE

SEQ ID NO: 19 - protein, 62 aa, synthetic construct
VELKREATLLELEAIEAAKAGDEEKRDELIKKLVELMKKLGLPQEQIDSKVEFIKNLAKKTK

SEQ ID NO: 20 - protein, 62 aa, synthetic construct
AKEAEEKAKKLEELIKEVEEELRKMAKEGKSEKELLDYANKKIPEKPAEATILVLKIVEEEK

SEQ ID NO: 21 - protein, 62 aa, synthetic construct
SEKVLEAKKKILNLESEISKKLGKLPEEVKELLKKTWEALEKDIEEAEKLIEEIKKKVEEIL

SEQ ID NO: 22 - protein, 62 aa, synthetic construct
KEEELKEFMEELREILEKKGLPEEEIEELLKKYKEELEKLIKSKNETEVEIFKAIKRQEALS

SEQ ID NO: 23 - protein, 62 aa, synthetic construct
SSENEKLLELFLNFYEKNVGTLTKEQKEHILKLAKETLNEELYKIFKEKMEEIEKKYKEEKA

SEQ ID NO: 24 - protein, 62 aa, synthetic construct
SSSKLEELKRVKEAIAKALEKALKTNPELAARLQEILDVLEEYLEAGKLDEAWKELGALLGS

SEQ ID NO: 25 - protein, 62 aa, synthetic construct
MEEKRKQLERGLAALEAAIEAGDKETAELYLRYIEYLASQDEELKAYVEARFAANPALKAYL

SEQ ID NO: 26 - protein, 62 aa, synthetic construct
SSLQALTERLFNEALELKEELKSLSPEEREKLIKERLEEVKKEDPENYPLFSRIVESMYKSL

SEQ ID NO: 27 - protein, 62 aa, synthetic construct
SSLRERAYRTLREAAAATPESERPAVAARLAELWERLSEENIEAVLAEAEALLAEQLARAAA

SEQ ID NO: 28 - protein, 62 aa, synthetic construct
STTTEQALAILARVAELVAKGLTPEDRESLAAARALAESVIASSSPEDAAKLRAALAELEAG

SEQ ID NO: 29 - protein, 62 aa, synthetic construct
SEELLELVKKYMKERIEKAPLEKLPEVLEKLKLLAERIGLSEEDIKKLMEEAKALIAKKKAA

SEQ ID NO: 30 - protein, 62 aa, synthetic construct
SAELEAIKARIRAEWDALGDEEGKEVMEKIFEYLLKNFPELTPEEIEQLLEQVRQSILAQRA

SEQ ID NO: 31 - protein, 62 aa, synthetic construct
SSLEQREKEFFEELDAMIAAGASLEELKAKVASFLRENPEISSETYNKLRARVKAYQAALAA

SEQ ID NO: 32 - protein, 62 aa, synthetic construct
MSDEEIEALVERIVASAQGLTEEQKAQLKAFLLELFKQRSSLSNSEILSLIREKVEALKAAA

SEQ ID NO: 33 - protein, 62 aa, synthetic construct
SAAAARRAELVQKIIDYLQKTLKALGKLEEAPKVIAAVQALVEAGASELELLRYAYQVREAL

SEQ ID NO: 34 - protein, 62 aa, synthetic construct
MTLAEIEAERQALLAEIREEGLSLAEAQKRILDWLLELYERTHNPELVSQLARDFVAALEAL

SEQ ID NO: 35 - protein, 62 aa, synthetic construct
RKFVTPESLKKYIEKNREKYEEVKKYMEALKKAGYMTPEVWKLFDELFEKIEKERELEKLLK

SEQ ID NO: 36 - protein, 62 aa, synthetic construct
SAAQAALAAELLARIEALRAEGASLEELAELLDEVRKALPLLTPEQQAEVIAAVRALLESFK

SEQ ID NO: 37 - protein, 62 aa, synthetic construct
SPEEERRRLQERLESYAAYLEAQIAAGVDPETRARYEAALAIIRESEDPEEAVEKLREFNAS

SEQ ID NO: 38 - protein, 62 aa, synthetic construct
SAAARRALLEARLAELEENLSKLPPEQAEQVLAYLKKSYPSMPPETIERFEAIIEQKKAELA

SEQ ID NO: 39 - protein, 62 aa, synthetic construct
SAELEQLRARALERAQTLSVEEIEELRTTLLALLRYRGAPEEEIAAVEAEFEAIIAAKRAAE

SEQ ID NO: 40 - protein, 62 aa, synthetic construct
SGAARAELIDAILREAQELLEAGAPLAEVEAWLRERAAAAGLSPETTAALLAWVRRRYEELA

SEQ ID NO: 41 - protein, 10 aa, synthetic construct
SGGSGGSGGS

SEQ ID NO: 42 - protein, 33 aa, synthetic construct
SGGSSGGSSGSETPGTSESATPESSGGSSGGSS

SEQ ID NO: 43 - DNA, 30 bp, synthetic construct
  source 1..30: mol_type = other DNA
agcggaggatccggaggatctggaggcagc

SEQ ID NO: 44 - DNA, 99 bp, synthetic construct
  source 1..99: mol_type = other DNA
tctggaggatctagcggaggatcctctggcagcgagacaccaggaacaagcgagtcagcaacaccagaaagcagtggcggcagttctggcggcagttct

SEQ ID NO: 45 - protein, 306 aa, synthetic construct
MALPVTALLLPLALLLHAARPDHWEEVFRWALEHLQEATQQNDPQKAKKILEEAHKWLRRELSEEEARAVVRWLKQLVDRELSTTTPAPRPPTPAPTIASQPLSLRPEACRPAAGGAVHTRGLDFACDIYIWAPLAGTCGVLLLSLVITLYCKRGRKKLLYIFKQPFMRPVQTTQEEDGCSCRFPEEEEGGCELRVKFSRSADAPAYQQGQNQLYNELNLGRREEYDVLDKRRGRDPEMGGKPRRKNPQEGLYNELQKDKMAEAYSEIGMKGERRRGKGHDGLYQGLSTATKDTYDALHMQALPPR

SEQ ID NO: 46 - protein, 45 aa, synthetic construct
TTTPAPRPPTPAPTIASQPLSLRPEACRPAAGGAVHTRGLDFACD

SEQ ID NO: 47 - DNA, 135 bp, synthetic construct
  source 1..135: mol_type = other DNA
accacgacgccagcgccgcgaccaccaacaccggcgcccaccatcgcgtcgcagcccctgtccctgcgcccagaggcgtgccggccagcggcggggggcgcagtgcacacgagggggctggacttcgcctgtgat

SEQ ID NO: 48 - protein, 39 aa, synthetic construct
IEVMYPPPYLDNEKSNGTIIHVKGKHLCPSPLFPGPSKP

SEQ ID NO: 49 - DNA, 117 bp, synthetic construct
  source 1..117: mol_type = other DNA
attgaggtgatgtatccacccccctatctggacaacgagaaatcaaatggcaccatcatccacgtaaagggcaagcacctgtgcccctctcctctgttccccggcccttccaagccc

SEQ ID NO: 50 - DNA, 189 bp, synthetic construct
  source 1..189: mol_type = other DNA
tccctggacgaggctaagaaactgctgcaagaggccgagaagctggctcgcaaactgaacgacagaatggaactggcctacgtggagttcctgaagcacatcctggagacagccaagaagcagaacgataagcgcaccatcgagagcgtgcgggacatggccagagacgccctggaagagctgcagagc

SEQ ID NO: 51 - DNA, 186 bp, synthetic construct
  source 1..186: mol_type = other DNA
gatcactgggaggaagtgttcagatgggccctggagcacctgcaagaggcgacccagcagaacgaccctcagaaagccaagaagatcctggaagaagctcacaagtggctccgccgcgagctgagcgaggaagaggcccgggccgtcgtgcggtggctgaagcagctggtggacagagagctgtcc

SEQ ID NO: 52 - DNA, 189 bp, synthetic construct
  source 1..189: mol_type = other DNA
agcgagaagatgaagaacatccaggagctgctggccgaggcggacaaatacctcgagaaggccaaggccgccaagaccaaggaggaggctaaagcctacctgagaaaggccgctgagaagctgctgcagtcccctctgagcggcctgcaagaggtggcctcccggatcctggaaaagctggagaaagag

SEQ ID NO: 53 - DNA, 189 bp, synthetic construct
  source 1..189: mol_type = other DNA
atgaagtctaagctgaagagctactccgaggccgccctgctgtacctgaccggcggtaaggagaagctggaactggccgagaagctgctgagcgaaatgtacgacctgttgggcgatgaggctgctaaagagcgcgccaagaagaacatcgaggagctgagaaaggaggaagaggaaaagctaaagaaa

SEQ ID NO: 54 - DNA, 189 bp, synthetic construct
  source 1..189: mol_type = other DNA
atggaagaggagaaagagaccagcgagtacatgagacagaccctgcacgagacactcgtggccatgggcctggatgagctggccctggaactgtactccgaggccaaggagaagggctggaacctgcaggagatcgtggacatgaacgacaagcgcctggctgccatcgccgccgaggaagccgctgct

SEQ ID NO: 55 - DNA, 189 bp, synthetic construct
  source 1..189: mol_type = other DNA
ggcgacaggaacattgcccgcatgatgaacttcatcaaggaaaagctggccgagctcagagccgaccccgctggtgctcctaaggccgaggccatcgagaagcggatggaagagatcagcaaggccctgaaagaggacttctccaccggcctggtgctgctgaatgagctgtacaaggagctcctggat

SEQ ID NO: 56 - DNA, 189 bp, synthetic construct
  source 1..189: mol_type = other DNA
atggaaaatctgatcaacgagtacaagaacgccgccgacgagctgtacaaaaaggccctggaaaagaaccctgatctggcgttcgagatcatcatggaagtgatcgacctcgaggaaaagaaagagacagtgaccgaggaggacattaaagagaagatcaagaagctgaaggaacgcctcgctctgctg

SEQ ID NO: 57 - DNA, 189 bp, synthetic construct
  source 1..189: mol_type = other DNA
ctggaagagaagttaaaagaggccgagaagaagctgaaagaaaccatcaagagcgtgggagtgtcccaggagacactggacgagatcaacaacataatcaagtctcagcacgcgaagctggctctgaacggcgtgggcgagggtgaatacgtcaaagtgctgaatgagctgatcgagaagatcaagaaa

SEQ ID NO: 58 - DNA, 189 bp, synthetic construct
  source 1..189: mol_type = other DNA
gacctgatggaacagatcgccagatccctgcgggatgagttcgtggcccgcttggaggccgagggcctgggccctgagctgatcgccgaggcgcgcgagagactggaaaaactgctgagcgtgctggaagcctctaccctgaagctgctgctggccgaggtggaagagtgggtcgcacggaagctggct

SEQ ID NO: 59 - DNA, 189 bp, synthetic construct
  source 1..189: mol_type = other DNA
atgcgcgaggaagagctgaagaagcggcgcgaggaagtgctgaagaaggtcgaggagctgaccaagctaggtggcaaggacctggaattcaaggccgagctggccgagcttctcgagaaagtggaagaaggcgacgaggaagctctgaaagagctggacagactgctggatgaggccttcaagaaactg

SEQ ID NO: 60 - DNA, 189 bp, synthetic construct
  source 1..189: mol_type = other DNA
tccatccctagcgagctgcagctgctcgctctgaagctgctggacttgaccgacaagctggctaaggacccctccgtggccaaagaggcgaaagaactgagagataagatcatcgaggccattcgctctggcgacgagaaggagctgctggaaatcaagaaagagcttgatgccttcctggccagcaag

SEQ ID NO: 61 - DNA, 189 bp, synthetic construct
  source 1..189: mol_type = other DNA
tccgacgccacccgccagctggagagcctgctggaccagatcgaggccttgctggccgccggcgacctggaagccgctacccagcagtggcaacagctggtggccctgctgggcgatctgagcgcggaggacctggagaagctgctgcctagaatccaggccgctcagcaggccttcatggccctgccc

SEQ ID NO: 62 - DNA, 186 bp, synthetic construct
  source 1..186: mol_type = other DNA
atggacaaggagaaagaaattgaggaacaggccaagaagctgaaagagatcgccgagaagctgaagaaagagctgggagcggatgagtccgaggtgaacctgatcgtggaactggccgtgaagcgcatcgagctgggcatgagcttcgaggacgctctgaaggaggccatcgagcagctgaagaag

SEQ ID NO: 63 - DNA, 186 bp, synthetic construct
  source 1..186: mol_type = other DNA
aacaaggccgaagaagagagagaaaagctgaaagaagaaatcaaagagatcatcgaggagctgatcaagaagaacccttccctgacccaggagacaatcgagaagatcaacagcaccctggaaaacctgatcctggcgggcgccagcaaggaggacatcatcaaggctctgaagaaagagatcgag

SEQ ID NO: 64 - DNA, 186 bp, synthetic construct
  source 1..186: mol_type = other DNA
gcggacgagctgcaggagaagctgaacaagctcaacgccctcatgctgaagtaccggaacagcagagccaccgagatctactacaatctggctctgaagctggaagaattggccaagacgggcaccgaagagaccaaggagaaggtgaagaaggccgaggaaaagctgaaagagtacgaggccaaa

SEQ ID NO: 65 - DNA, 186 bp, synthetic construct
  source 1..186: mol_type = other DNA
tcctctgcggaataccaggctctgcttgagcagaagcggctggaggccagaagactgctggccgaggccctgctgaagggcagcgaggagttgaaagagaagctgaaggagaagctgaaagagtggcgcgaggaaggcttccctgaggaactgatcaaggagctggaagaagagctggaaaaggcc

SEQ ID NO: 66 - DNA, 186 bp, synthetic construct
  source 1..186: mol_type = other DNA
ctactggaagagttcaagaaagagttggacgaactgctggagaagatcaagagcggcgaggtcactgaagaggatctgctgaagaagaccgaggaagctatcgaggaagtgaagaagctgcctaacgccgaaaagtaccagaccgagctgaaacgcctggtggccgaggccctcctgaagctgtcc

SEQ ID NO: 67 - DNA, 186 bp, synthetic construct
  source 1..186: mol_type = other DNA
gaggaagaggagcagaaaaagaacctgctgaagcagaagctgaagatcaaggccgagttcctgatcgagaagaccggcgacaaggagaaggtgctggagctggaaaagaagtacatcgaggctctggatagcggcaagaacaaagaagaagccgagaagctgctgaaagagatggaatccctcgaa

SEQ ID NO: 68 - DNA, 186 bp, synthetic construct
  source 1..186: mol_type = other DNA
gtggaactgaagcgcgaggccaccctgctcgaactggaagccatcgaggccgccaaggccggcgacgaggagaagagagatgagctgatcaagaaattggtcgagctgatgaagaagctgggcctccctcaggagcagatcgacagcaaggtggaattcatcaagaacctggctaagaagaccaag

SEQ ID NO: 69 - DNA, 186 bp, synthetic construct
  source 1..186: mol_type = other DNA
gccaaagaggccgaggaaaaggccaagaagctggaagagctgatcaaggaggtggaagaagagttgagaaagatggccaaggagggcaagagcgagaaagagctgctggactacgccaacaagaaaatccccgagaagcctgccgaagcgaccatcctggtgctgaagattgtggaggaggagaag

SEQ ID NO: 70 - DNA, 186 bp, synthetic construct
  source 1..186: mol_type = other DNA
tccgagaaggtgctggaggccaagaagaagattctgaacctggagagcgagatcagcaagaaactgggcaagctgcctgaggaggtgaaggagctgctgaaaaagacctgggaggctctggaaaaggacatcgaggaggccgagaagctgatcgaggaaatcaagaagaaagtcgaagagatcctg

SEQ ID NO: 71 - DNA, 186 bp, synthetic construct
  source 1..186: mol_type = other DNA
aaggaggaagaactgaaagagttcatggaagaactgagagagatcctggagaagaagggcctgcctgaggaagagattgaggaactgctgaagaagtacaaggaggagctggaaaagctgatcaagagcaagaacgagaccgaggtggaaatcttcaaagccatcaagcgccaggaggctctgtcc

SEQ ID NO: 72 - DNA, 186 bp, synthetic construct
  source 1..186: mol_type = other DNA
tccagcgagaacgagaaactgctggaactgtttctgaacttctacgagaagaacgtgggcaccctaaccaaggaacagaaggaacacatcctgaaactggctaaggagacactgaacgaggagctgtacaagatcttcaaggaaaagatggaagagatcgagaagaagtacaaggaggaaaaggcc

SEQ ID NO: 73 - DNA, 186 bp, synthetic construct
  source 1..186: mol_type = other DNA
tccagcagcaagctggaggaactgaagcgggtcaaagaggccatcgccaaggcgctcgagaaggccctgaagaccaaccctgagctggccgccagactgcaggaaatcctggacgtgctggaagagtacctggaagctggcaagctggatgaggcctggaaggagcttggagctctgctgggctct

SEQ ID NO: 74 - DNA, 186 bp, synthetic construct
  source 1..186: mol_type = other DNA
atggaagagaagcggaagcagctggaacgtggtctggccgctctggaggctgccatcgaggccggcgacaaggaaaccgccgagctgtacctgaggtacatcgagtacctggccagccaggacgaggaactgaaggcctacgtggaagccagattcgccgccaaccctgcgctgaaagcctatctg

SEQ ID NO: 75 - DNA, 186 bp, synthetic construct
  source 1..186: mol_type = other DNA
tccagcctgcaggccctgaccgagcgcttattcaacgaggctctggaactgaaagaggagctgaagtctctgagccctgaggaacgcgagaagctgatcaaggagcggctggaagaagtgaagaaagaggacccggagaactaccccctgttcagcagaatcgtggaatccatgtacaagagcctc

SEQ ID NO: 76 - DNA, 186 bp, synthetic construct
  source 1..186: mol_type = other DNA
tccagcctgagagagcgggcctaccggaccttgcgcgaagctgctgccgccacacccgaatctgagcgccctgccgtggccgctagactcgccgagctgtgggagagactgagcgaggaaaacatcgaggccgtgctggctgaggctgaagctctgctggcagagcagctggctagagctgcagct

SEQ ID NO: 77 - DNA, 186 bp, synthetic construct
  source 1..186: mol_type = other DNA
tccacaaccaccgagcaggccctggccatcctggctagagtggccgaactggtcgctaagggactgacacctgaggatagagagagcctggctgctgcgagagcactcgctgaatctgtgatcgccagcagctctcctgaggatgctgctaagctgagagccgctctggccgagctggaagccgga

SEQ ID NO: 78 - DNA, 186 bp, synthetic construct
  source 1..186: mol_type = other DNA
tccgaggaactgctcgagctggtcaagaaatacatgaaggaacgcatcgagaaggcccctctggaaaagttgcccgaagtgctggaaaagctgaagctgctggccgagcggatcggcctgagcgaggaggacattaagaagctgatggaagaggccaaggccctgatcgccaagaaaaaagctgct

SEQ ID NO: 79 - DNA, 186 bp, synthetic construct
  source 1..186: mol_type = other DNA
tccgcggagctcgaggccatcaaggccagaattagagccgagtgggatgccctgggcgacgaggaaggaaaagaggtgatggaaaagatcttcgagtacctgctgaagaacttccccgagctgacccctgaggagatcgagcagctgctggaacaggtgcggcagagcatcctggcccagcgcgct

SEQ ID NO: 80 - DNA, 186 bp, synthetic construct
  source 1..186: mol_type = other DNA
tcctcgctcgagcagcgcgagaaagagttcttcgaggaactggacgccatgatcgccgctggcgccagcctggaagagctgaaggccaaggtggcatcttttctgcgggaaaaccctgagatcagcagcgagacctacaacaagctgagagccagagtgaaggcctaccaggccgccctggctgct

SEQ ID NO: 81 - DNA, 186 bp, synthetic construct
  source 1..186: mol_type = other DNA
atgagcgacgaggaaatcgaggccctggtcgagcggatcgtggcctctgcccagggcctgaccgaggagcagaaggctcagctgaaagccttcctgctggaactgttcaagcagcgctcctccttgagcaacagcgagattctctctctgatcagagagaaggtggaagctctgaaggcggcagcc

SEQ ID NO: 82 - DNA, 186 bp, synthetic construct
  source 1..186: mol_type = other DNA
tccgccgctgctgcacgccgtgccgagctggtccagaagatcatcgactacctgcagaaaaccctgaaggccctgggcaagctggaagaggcccccaaggtgatcgccgccgtgcaggctctggtggaagccggagccagcgagctcgagctgctgagatacgcctaccaggtgcgggaggccttg

SEQ ID NO: 83 - DNA, 186 bp, synthetic construct
  source 1..186: mol_type = other DNA
atgaccttggccgagatcgaggccgagagacaggccctgctcgctgagattcgcgaggaaggcctgagcctggctgaggcccagaagcggatcctggactggctgctggaactgtacgagcgcacacacaaccctgagctggtgtcccagctggccagagatttcgtggccgctctggaagcgctc

SEQ ID NO: 84 - DNA, 186 bp, synthetic construct
  source 1..186: mol_type = other DNA
cggaagttcgtgacccctgagagcctgaagaagtacatcgagaagaaccgcgagaagtacgaggaagtcaagaaatacatggaagccctgaagaaggccggctacatgacccccgaggtgtggaagctgttcgacgagctgttcgagaagatcgagaaagagagagagctggaaaagctgctgaaa

SEQ ID NO: 85 - DNA, 186 bp, synthetic construct
  source 1..186: mol_type = other DNA
tctgccgcccaggccgctctggccgctgaattgctggccagaatcgaggcactgagagctgaaggcgctagcctggaagagctagctgagctgctggacgaggtgcggaaggcactgcctctgctgacccccgagcagcaggccgaggtgatcgctgccgtccgcgcacttctcgagtccttcaag

SEQ ID NO: 86 - DNA, 186 bp, synthetic construct
  source 1..186: mol_type = other DNA
tccccggaggaagagcggcgccgtctacaggagagactggaaagctacgccgcctacctggaagcccagatcgccgctggcgtggatcctgagaccagagcccggtacgaggctgctctggccatcatcagagagagcgaggaccccgaggaggccgtggaaaagctgcgcgagttcaacgcctct

SEQ ID NO: 87 - DNA, 186 bp, synthetic construct
  source 1..186: mol_type = other DNA
tctgccgctgctcgcagggccctgctggaagcgagactggccgagctggaagagaacctgagcaagctgcctccagagcaggccgaacaggtgctggcctacctgaagaagtcctaccccagcatgcctcccgaaaccatcgagcggttcgaggccatcatcgagcagaaaaaggcggagctcgct

SEQ ID NO: 88 - DNA, 186 bp, synthetic construct
  source 1..186: mol_type = other DNA
tccgccgagctcgagcagctacgcgcgagagctctggaacgcgctcagacactgagcgtggaagagatcgaggagctgcggaccaccctgctggccctgctgagatacagaggcgcccctgaggaagagattgccgccgtggaagccgagttcgaggccatcatcgccgcgaagcgggccgctgag

SEQ ID NO: 89 - DNA, 186 bp, synthetic construct
  source 1..186: mol_type = other DNA
tccggcgccgccagagccgagttgatcgacgccatcttgcgcgaggcccaggagctgctggaagcaggagctcctctggcagaggtggaagcctggctgagagagagagctgcagctgctggactgagccctgagacaaccgctgctctgctggcttgggtcagaaggagatacgaggaactggcg

SEQ ID NO: 90 - DNA, 918 bp, synthetic construct
  source 1..918: mol_type = other DNA
atggccctgcccgtgaccgccctgctgctgcccctggccctgctgctgcacgccgccaggcccgatcactgggaggaagtgttcagatgggccctggagcacctgcaagaggcgacccagcagaacgaccctcagaaagccaagaagatcctggaagaagctcacaagtggctccgccgcgagctgagcgaggaagaggcccgggccgtcgtgcggtggctgaagcagctggtggacagagagctgtccaccactaccccagcaccgaggccacccaccccggctcctaccatcgcctcccagcctctgtccctgcgtccggaggcatgtagacccgcagctggtggggccgtgcatacccggggtcttgacttcgcctgcgatatctacatttgggcccctctggctggtacttgcggggtcctgctgctttcactcgtgatcactctttactgtaagcgcggtcggaagaagctgctgtacatctttaagcaacccttcatgaggcctgtgcagactactcaagaggaggacggctgttcatgccggttcccagaggaggaggaaggcggctgcgaactgcgcgtgaaattcagccgcagcgcagatgctccagcctaccaacaggggcagaaccagctctacaacgaactcaatcttggtcggagagaggagtacgacgtgctggacaagcggagaggacgggacccagaaatgggcgggaagccgcgcagaaagaatccccaagagggcctgtacaacgagctccaaaaggataagatggcagaagcctatagcgagattggtatgaaaggggaacgcagaagaggcaaaggccacgacggactgtaccagggactcagcaccgccaccaaggacacctatgacgctcttcacatgcaggccctgccgcctcgg

SEQ ID NO: 91 - protein, 18 aa, synthetic construct
GSTSGSGKPGSGEGSTKG

SEQ ID NO: 92 - DNA, 54 bp, synthetic construct
  source 1..54: mol_type = other DNA
ggaagcacgtccggctcagggaagccgggctccggcgagggaagcacgaagggg